European Patent Specification EP 3 552 632 B1, published July 12, 2023. Title: PHARMACEUTICAL COMPOSITION FOR TREATING AND PREVENTING CHRONIC DISEASES. Applicant: STELIC INSTITUTE & CO., INC. The sequence listing filed with the application follows.

SEQUENCE LISTING (6 sequences)

SEQ ID NO: 1 - RNA, 25 nt, Artificial Sequence
  An artificially synthesized siRNA sequence
gauuguauucaucuugcucugcucc

SEQ ID NO: 2 - RNA, 25 nt, Artificial Sequence
  An artificially synthesized siRNA sequence
ggagcagagcaagaugaauacaauc

SEQ ID NO: 3 - RNA, 27 nt, Artificial Sequence
  An artificially synthesized siRNA sequence
gauuguauucaucuugcucugcuccau

SEQ ID NO: 4 - RNA, 27 nt, Artificial Sequence
  An artificially synthesized siRNA sequence
ggagcagagcaagaugaauacaaucag

SEQ ID NO: 5 - DNA, 4813 bp, Homo sapiens
  CDS (614)..(2299): NM_015892.4: Homo sapiens carbohydrate sulfotransferase 15 (CHST15), transcript variant 1, mRNA
gaggcggcgtgactcgggagttgccggcgcttcccggcggtggcggcgtctctggccggccttggtgcggcgagccgagcgaggcagctctgagccgcgcggaaatctggcattttttaaagtttgcgccccacaaagaggaaatattccaaaggtactcaggatgtaaaaggggagatcttcacagatgcctccgtggatggcatggcaatccatccatcaatgagaagaccatgatttcttttaattttctgtgtgtttccacattccccagtgagaattcttccacctttttttgtgccatgggaaaaacctgaagggcaggcagagctgctcccgaacttgtgaccttctctgaggttgcagcggctcttgtagaacatgactctgggacatcacttccttttgttttctttcggagctgaaccaaagaatgtgcaccctctttctctagtgctgtggtgtctgcttatttttgtatttgtgctttccatccatcttctgtgatcacaaggcattcttaaggttttctagcacgacttgcggacatccagactcgtggggggcccacccatggctcggtaagccagcagcccagggcactggcactaccatgaggcactgcattaattgctgcatacagctgttacccgacggcgcacacaagcagcaggtcaactgccaagggggcccccatcacggtcaccaggcgtgccccacgtgcaaaggagaaaacaaaattctgtttcgtgtggacagtaagcagatgaacttgcttgctgttctcgaagtgaggactgaagggaacgaaaactggggtgggtttttgcgcttcaaaaaggggaagcgatgtagcctcgtttttggactgataataatgaccttggtaatggcttcttacatcctttctggggcccaccaagagcttctgatctcatcacctttccattacggaggcttccccagcaaccccagcttgatggacagcgaaaacccaagtgacacaaaggagcatcaccaccaatcctctgtaaataatatttcatacatgaaggactatccaagcattaaattaattatcaacagcatcacaactaggattgagttcacgaccagacagctcccagacttagaagaccttaagaagcaggagttgcatatgttttcagtcatccccaacaaattccttccaaacagtaagagcccctgttggtacgaggagttctcggggcagaacaccaccgacccctacctcaccaactcctacgtgctctactccaagcgcttccgctccaccttcgacgccctgcgcaaggccttctggggccacctggcgcacgcgcacgggaagcacttccgcctgcgctgcctgccgcacttctacatcatagggcagcccaagtgcgggaccacagacctctatgaccgcctgcggctgcaccctgaggtcaagttctccgccatcaaggagccacactggtggacccggaagcgctttggaatcgtccgcctaagagatgggctgcgagaccgctatcccgtggaagattatctggacctctttgacctggccgcacaccagatccatcaaggactgcaggccagctctgcaaaggagcagagcaagatgaatacaatcattatcggggaggccagtgcctccacgatgtgggataataatgcctggacgttcttctacgacaacagcacggatggcgagccaccgtttctgacgcaggacttcatccacgcctttcagccaaatgccagactgattgtcatgctcagggaccctgtggagaggttgtactcagactatctctactttgcaagttcgaataaatccgcggacgacttccatgagaaagtgacagaagcactgcagctgtttgaaaattgcatgcttgattattcactgcgcgcctgcgtctacaacaacaccctcaacaacgccatgcctgtgaggctccaggttgggctctatgctgtgtaccttctggactggctcagcgtttttgacaagcaacagtttctcattcttcgcctggaagatcatgcatccaacgtcaagtacaccatgcacaaggtcttccagtttctgaacctagggcccttaagtgagaagcaggaggctttgatgaccaagagccccgcatccaatgcacggcgtcccgaggaccggaacctggggcccatgtggcccatcacacagaagattctgcgggatttctacaggcccttcaacgctaggctggcgcaggtcctcgcggatgaggcgtttgcgtggaagacgacgtgagagctgaattgttgctgcacgtgctgggcccgccaatgccgtcatcatcaggattttacaaatctctttgcggggaactgtttcactcatggtatggaaaaccccaggactctgccactctaggcacacatgaattataaccattttggaatttccttcgtgatgttcgagagctcagcaatggacccctcacagagctcctctatccgaggccattggagaccccagtttctcaagaattcagctctgctctgagcgtcctggagcttggggatgcagccagctggcctgcactgggtgtggagagaacacctagggaaggcagcctggccctgcccgcctccgccttctggagagcctctgggttctgagtcagcaagccagaggtcatgccacaggcctggctggaacttacacttcacgttccctttttttccccctagagatggggtctcgccgtgttgcacagactgtctgtattcaatggctatcttcacaggtgtgatcataccacattcacttctgaaacactcttgttgcgatcgctaacctcactgggacagagaaccgcagtctttcgagaatggaggctcttcattttttttttctcctttactccaaactcagccctccagtttcttcagatgtaaaccctgttaacgtcactgtttccaaaaggaaaaaaataagtcagtttttggcagcaccttcatctttctgacctcctcctattctgtccttgtggacttatgtttaacatagaaaatgaatgcgtttaaaacaaaaccactttctgcatttaaccagtcctggctctctctctgctgcctcttcatacgttttctcaagaacttcagtttataattggaagagaaatttttgctgttaatgccagaatgagcaacctcaaggaattgaacacttcttggaaaatctaggtaattcaagccctcatcaggtttacaagatcatcagagaaacagaggattttaatttttagttctggccggctacaggctccatttctctgccttcccattggaaatagtttatttccacattctccactgcgtgtggtcaaagttcctcacccagcaagggactatagatactcgtgtcccaattccaaaacacaatgcacaagctgaacttgggctgaacgtggcgtgttgagatttggaatgaggtttctaagagccgtgttcttcatggaattttccaggccacttggcagcttggtttaccgatggatgggctagagatcttgtcgtttcttggaagtcacagggaagattgaagagaacgcttgagcatccttggcaacagcccaggtgggacctggatgaagctttgcactcaagtattgtcaagggaagcttcctgtgaaccaaagttctcaggccaaggtctcgcccaccaaagccagaaagtgcaagcacccgtctacccagctctaacttgtatgtgtgagacagaccaggcttcgggggtaggaggatctgcagttgttcagccgtctttctgctggtgttgtctttctgccatcagagaagggacacacagcccgttcgaaggtgtgcagagggctctgagcgccaggatggccagggctgtttttgctactgaaggagcgtgtgtcctgaactcccacttgcagggacagtccccaccttctctatagccggcactgggagcagccgccagcagggaaatctggcctgagcacaaggatgctttagggagagatcacttcagtgtgtgtgtatatttatttgcagtacagtgcgcgcgtgtgtgtgtgtgtacgcgcacgtgtgggtgagtgcgtcttctgagtgggttctgttcagttgctaatgaggctcctccgctctggacacaacccttttatagattaatttctctgccaattaacttgtcattttcagtacatattttactattccacaccaaccataattacaacaagggatttttcttatgcactcctatgcatgtgaataacatgtggtgtaattctgcttcttacagaagtattactgaaggtattatttccaatattatttggtttattatgcggatcttttttatatatgcagtcccatcccttctgtgccactcaatgccatccagacatggtttttccctccaggggcctttctctccagagggcacttcggctgcctctgcttcctctcattcgaggcccggctcttgctgacagaataggttccgttctgggcggtggttctcgagcctgccattcaaaaccaaagcaaattggagcatttctcacaacatggtattgaagttcctttttgttctcaaaagttgtgaccgtgttaaattgtactcccttagtcctgtaaggtatgttaagtgaatcgcagttacgctgtacttttattaatatttaacataattaaagatggacccataagagtgacgcctgtggagcgcgtgctcttcctctgcagccaagcaaaaaaaaaaaaaaaaaaaaaaaaaaaaaaa

SEQ ID NO: 6 - protein, 561 aa, Homo sapiens
MRHCINCCIQLLPDGAHKQQVNCQGGPHHGHQACPTCKGENKILFRVDSKQMNLLAVLEVRTEGNENWGGFLRFKKGKRCSLVFGLIIMTLVMASYILSGAHQELLISSPFHYGGFPSNPSLMDSENPSDTKEHHHQSSVNNISYMKDYPSIKLIINSITTRIEFTTRQLPDLEDLKKQELHMFSVIPNKFLPNSKSPCWYEEFSGQNTTDPYLTNSYVLYSKRFRSTFDALRKAFWGHLAHAHGKHFRLRCLPHFYIIGQPKCGTTDLYDRLRLHPEVKFSAIKEPHWWTRKRFGIVRLRDGLRDRYPVEDYLDLFDLAAHQIHQGLQASSAKEQSKMNTIIIGEASASTMWDNNAWTFFYDNSTDGEPPFLTQDFIHAFQPNARLIVMLRDPVERLYSDYLYFASSNKSADDFHEKVTEALQLFENCMLDYSLRACVYNNTLNNAMPVRLQVGLYAVYLLDWLSVFDKQQFLILRLEDHASNVKYTMHKVFQFLNLGPLSEKQEALMTKSPASNARRPEDRNLGPMWPITQKILRDFYRPFNARLAQVLADEAFAWKTT